European Patent Application EP 4 582 538 A1, published July 9, 2025. Title: MONOOXYGENASE MUTANT AND USE THEREOF. Applicant: ASMCHEM LABORATORIES TORIES(TIANJIN)CO.,LTD. The sequence listing filed with the application follows.

SEQUENCE LISTING (1 sequence)

SEQ ID NO: 1 - protein, 564 aa, Rhodococcus jostii
MTTSMKAANPMNFPSTSDTGIVDVLGVGAGFSGLYLSHRLTTAGWTFAGFEAGPSVGGTWFWNTYPGARCDVESIYYSYSFDEALQQEWTWSQRFAPQAEILSYINHVADRFDLRKHFTFNTRVVGATWNAAERLWEVQLDNGETRRGRYLISGAGGLSTPKDFDVPGLGNFTGLQVSTSRWNISLDDLAGKRVAVIGTGSSGVQAIPLIAEVAEHVTVFQRTPNYVMPARNAELPLERVDSIKDDYPAIREECRHSPGGIPDRPVTDKAFDVSAEERQRRYEAAYERSGFNGVGGEFADLLTDVEANRTASEFIHDKIREIVEDPATAELLVPRYHPLGAKRSVFGTDYYETYNRPNVSLVSLRDEPIETMTANAIVTSKGTYEADAVVLAIGFDAFTGPLYGLGLTGASGRKLQETWQDGIRTYLGMMTTDFPNFFMVAGPQSPALASNVVMTIEQAVDWIADLIEHARDSGATLVEATPEGQNDWVDITEETVAQTLYATTDSWYRGSNVEGKPNTFMGYVGGVGKYRRMCTEIAKRGYPGVRIDGETESPHLGPIHREIS